European Patent Specification EP 3 282 016 B1, published August 20, 2025. Title: Resistenzgen gegen Wurzelbärtigkeit. Applicant: KWS SAAT SE. The sequence listing filed with the application follows.

SEQUENCE LISTING (6 sequences)

SEQ ID NO: 1 - DNA, 2784 bp, Beta vulgaris subsp. vulgaris
atggaagcatttcagtctgacatcgcgttggctttgcttcaagatttgttagaaagatttaaatcattagtcattgatgaagcaggtcaaatagtacagtttgatgcagaggatgaactgaagaaactggagaggaagctattaaaggcccaagtcttgcttggcagctttcagctgacaaccgacaaaaattggcaacactgggttggtgatgtcaccagagtttgctatgatgctgaagacttggttgatgatatagtgcttgatgccggcaaaacttcattgcttgagaagatcttgtcatatttcacaagaggaagcatggcccggaagatccaagagctccaagataggttggaagatataataagtggattagacatggttaacaaaacaaagcaacgagcacagcaatgttatttaggggagtttgtttatggtaacgaacaattactcctaacagagaagttatttgggagggatgcagataaggagaacattatctcgatgttactggaacagacaataagctcagtatctattgttggcatggacgggcttggtaaaacaacacttgctcagaatatgctatatgattccagaatccaggagaaatttcatcatagagtgtgggtccgtgtgtctgcgaagtttgatctgagaaaaatcacagactttatcttacatcgcaggcaggaatgtgagtacagctttcttcctgagaaaatatatggtttgtttcacgatctgtatatgggtaaaagtatattgattgtgttggatgacttatgggatgtgaagtacgatgattggaggtcttttcgctctttgtttctgcgctcttctggttgcaaagttcttctcaccactagcaatccaaatgtaacaacggttacaaaagctacaccgtatcatttaaaattgatgaaggatgaagattgccaagctctaatcatggatagagttttctcatctaataatctatctgaacgtcagcttgtaatcttggaggatattgctgtagcagttgcccaaaagtgcaagggcttgcctctggcagccaatgttttgggcctccatttatcttctgggcgtagagatgatgaatggatgaattttttagatagagacatatgcgagttgagggtattcaaagaagaaatatttcctgcttttagactgaacaacccttgtttggcatcacacttaaagaagtgtcttgcttactgctcattatttcctcatgattacgatttcaagaaagaaaacttagttcagctatggatgtcagaaggtttttttctgcctcaaaggatgacaagcctagaacaaattggcagtgattgttttgatgagctcttgtggagatctgtctttcaactttcacatgttggtgatcaggagctaccaacttacaaaatgcatgaatttattcgcaggtttgctgaatttgtggcctcagacacatgtttccggtgggaggaaggtcagagctctttctcagttccttggtacaaaacggctcgtcatttatctttgctttgtgattgcatcaaaccagcattccttaaatacattgaaaattgtgatggtctgaggacatttcttctgctaagtgaaaaaggaacacaaattggccagcttccttattcacttttccagaaactagtacgactgcgagttctggacttgagtcgtactgatattgatgagctcccggagtcattgggtagattaaagtatcttcggtatttcgatgcatctcagacacatatcctaaggttgcctaagtcagtgaccaaccttcatcaattacaagtactcagattgagagaatgttataaacttctagagttgccaaaaaacattaagaacctgactaaccttctacatcttgacgtggacattaaaggattgaggtgtaggccagcaagtataggaagtctaagttgccttaaaacacttccttcctttgctgtttgtaagaaggtaggatatcgcattgcagagttgaagaatctgaagaatctatgtggtacaatttgccttagtaatcttgaaaatgttaaggatggggcagaggccagggacgcgatgatatgtgataagccatatatcaaaaggttggaattagaatggagccgtttttctcgagatgggtcaatagagatggatgttcttgctggccttcaaccagacaaaaatttgaaagaactgcaagtaatcaactatggtggttcgagctttcctgcttggcttacaagcccatcttgcatgcttgtgagtatctatatgcaaaattgtcggcaagatgactttctgccttcacttgggcaacttcctttcctcaagacacttcatgttgaaggtatgcatagcgtgaagtatgtggactatcatttttgtggtgaaagtacaactggggcctttccttccttggaatcactgaagatccaggacatgatgtgccttatgagttggtatccattaccagacaatagcttgctccaactccgtgatcttacaatagaggattgtccaagtctcttctcaatgcaatcgctaaaacatatgagttcactacaagaactagtgatcaactgttgcccagggctggagacattgcctcagctaccaggatcaattcagtcattgatcattttcgaaagtgatatggtgaaacagcggtgtcagattgaagaaggtcctgaatggaacatcataaaaacaattccttatgtggagattgactacgagagtatgtttcctggagattcaagttag

SEQ ID NO: 2 - protein, 927 aa, Beta vulgaris subsp. vulgaris
MEAFQSDIALALLQDLLERFKSLVIDEAGQIVQFDAEDELKKLERKLLKAQVLLGSFQLTTDKNWQHWVGDVTRVCYDAEDLVDDIVLDAGKTSLLEKILSYFTRGSMARKIQELQDRLEDIISGLDMVNKTKQRAQQCYLGEFVYGNEQLLLTEKLFGRDADKENIISMLLEQTISSVSIVGMDGLGKTTLAQNMLYDSRIQEKFHHRVWVRVSAKFDLRKITDFILHRRQECEYSFLPEKIYGLFHDLYMGKSILIVLDDLWDVKYDDWRSFRSLFLRSSGCKVLLTTSNPNVTTVTKATPYHLKLMKDEDCQALIMDRVFSSNNLSERQLVILEDIAVAVAQKCKGLPLAANVLGLHLSSGRRDDEWMNFLDRDICELRVFKEEIFPAFRLNNPCLASHLKKCLAYCSLFPHDYDFKKENLVQLWMSEGFFLPQRMTSLEQIGSDCFDELLWRSVFQLSHVGDQELPTYKMHEFIRRFAEFVASDTCFRWEEGQSSFSVPWYKTARHLSLLCDCIKPAFLKYIENCDGLRTFLLLSEKGTQIGQLPYSLFQKLVRLRVLDLSRTDIDELPESLGRLKYLRYFDASQTHILRLPKSVTNLHQLQVLRLRECYKLLELPKNIKNLTNLLHLDVDIKGLRCRPASIGSLSCLKTLPSFAVCKKVGYRIAELKNLKNLCGTICLSNLENVKDGAEARDAMICDKPYIKRLELEWSRFSRDGSIEMDVLAGLQPDKNLKELQVINYGGSSFPAWLTSPSCMLVSIYMQNCRQDDFLPSLGQLPFLKTLHVEGMHSVKYVDYHFCGESTTGAFPSLESLKIQDMMCLMSWYPLPDNSLLQLRDLTIEDCPSLFSMQSLKHMSSLQELVINCCPGLETLPQLPGSIQSLIIFESDMVKQRCQIEEGPEWNIIKTIPYVEIDYESMFPGDSS

SEQ ID NO: 3 - DNA, 2784 bp, Beta vulgaris subsp. maritima
atggaagcatttcagtctgacatcgcgttggctttgcttcaagatttgttagaaagatttaaatcattagtcatcgatgaagcaggtcaagtagtacagtttgatgcagaggatgaactgaagaaactggagaggaagctaaaaaaggcccaagtcttgcttggcagctttcagctgacaaccgacaaaaattggcaacactgggttggtgatgtcaccagagtttgctatgatgctgaggacttggttgatgatatagtgcttgatgccggcaaaacttcattgcttgagaagatcttgtcatatttcacaagaggaagcatggcccggaagatccaagagctccaagataggttggaagatataataagtggattagacatggttaacaaaacaaagcaacgagcacagcaatgttatttaggggagtttgtttatggtaacgaacaattactcctaacagagaagttatttgggagggatgcagataaggagaacattatcacgatgttgctggaacagacaataagctcagtatctattgttggcatggacgggcttggtaaaacaacacttgctcagaatatactatatgattccagaatccaggagaaatttcatcatagagtgtgggtccgtgtgtctgcgaagtttgatctgagaaaaatcacagactttatcttacatcgcaggcaggaatgtgagtacagctttcttcctgagaaaatacattgtttgtttcacgatctgtatatgggtaaaagtatattgattgtgttggatgacttatgggatgtgaagtacaatgattggagctcttttcgctctttgtttctgcgctcttctggttgcaaagttcttctcaccactagcaatccaaatgtaacaacggttacaaaagctactccgtatcatttacaattgatgaaggatgaagattgccaagctctaatcatggatagagttttctcatctaataatctatctgaacgtcagcttgtaatcttggaggatattgctgtagcagttgcccaaaagtgcaagggcttgcctctggcagccaatgttttgggcctccatttatcttctgggcgtagagatgatgaatggatgaattttttagatagagacatatgtgagttgagggtattcaaagaagaaatatttcctgcttttagactgaacaaccctggtttggcatcacacttaaagaagtgtcttgcttactgctcattatttcctcatgattacgatttcaagaaagaaaacttagttcagctatggatgtcagaaggtttttttctgcctcgaaggatgacaagcctagaacaaattggcagtgattgttttgatgagctcttgtggagatctgtctttcaactttcacatgttggtgatcaggagctaccaacttacaaaatgcatgaatttattcgcaggtttgctgaatttgtggcctcagacacatgtttccggtgggaggaaggtcagagctctttctcagttccttggtacaaaacggctcgtcatttatctttgctttgtgattgcatcaaaccagcattccttaaatacattgaaaattgtgatggtcttaggacatttcttctgctaagtgaaaaaggaacacaaattggccagcttccttattcacttttccagaaactagtacgactgcgagttctggacttgagtcatactgatattgatgagctcccggagtcattgggtagattaaagtatcttcggtatttcgatgcatctcagacacatatcctaaggttgcctaagtcagtgaccaaccttcatcaattacaagtactcagattgagagaatgttataaacttctagagttgccaaaaaacattaagaacctgactaaccttctacatcttgacgtggacattaaaggattgaggtgtaggccagcaagtataggaagtctaagttgccttaaaacacttccttcctttgctgtttgtaagaaggtaggatatcgcattgcagagttgaagaatctgaagaatctatgtggtacaatttgccttagtaatcttgaaaatgttaaggatggggcagaggccagggacgcgatgatatgtgataagccatatatcaaaaggttggaattagaatggagccgtttttctcgagatgggtcaatagagatggatgtccttgctggccttaaaccagacaaaaatttgaaagaactgcaagtaatcaattatggtggttcgagctttcctgcttggcttacaagcccatcttgcatgcttgtgagtatctatatgcaaaactgtcggcaagatgactttctgccttcgcttgggcaacttcctttcctcaagacacttcatgttgaaggtatgcatagcgtgaagtatgtggactatcatttttgtggtgaaagtacaactggggcctttccttccttggaatcactgaagatccaggacatgatgtgccttatgagttggtatccattatcagacaatagcttgctccagctccgtgatcttacaattgaggattgtccaagtctcttctcaatgcaatcgctaaaacatatgagttcactacaagaactagtgatcaactgttgcccagggctggagacattgcctcagctaccaggatcagttcagtcattgatcattttcggaagtgatatggtgaaacagcggtgtcagattgaagaaggtcctgaatggaacatgataaaaacaattccttatgtggagattgactacgagagtatgtttcctggagattcaagttag

SEQ ID NO: 4 - protein, 927 aa, Beta vulgaris subsp. maritima
MEAFQSDIALALLQDLLERFKSLVIDEAGQVVQFDAEDELKKLERKLKKAQVLLGSFQLTTDKNWQHWVGDVTRVCYDAEDLVDDIVLDAGKTSLLEKILSYFTRGSMARKIQELQDRLEDIISGLDMVNKTKQRAQQCYLGEFVYGNEQLLLTEKLFGRDADKENIITMLLEQTISSVSIVGMDGLGKTTLAQNILYDSRIQEKFHHRVWVRVSAKFDLRKITDFILHRRQECEYSFLPEKIHCLFHDLYMGKSILIVLDDLWDVKYNDWSSFRSLFLRSSGCKVLLTTSNPNVTTVTKATPYHLQLMKDEDCQALIMDRVFSSNNLSERQLVILEDIAVAVAQKCKGLPLAANVLGLHLSSGRRDDEWMNFLDRDICELRVFKEEIFPAFRLNNPGLASHLKKCLAYCSLFPHDYDFKKENLVQLWMSEGFFLPRRMTSLEQIGSDCFDELLWRSVFQLSHVGDQELPTYKMHEFIRRFAEFVASDTCFRWEEGQSSFSVPWYKTARHLSLLCDCIKPAFLKYIENCDGLRTFLLLSEKGTQIGQLPYSLFQKLVRLRVLDLSHTDIDELPESLGRLKYLRYFDASQTHILRLPKSVTNLHQLQVLRLRECYKLLELPKNIKNLTNLLHLDVDIKGLRCRPASIGSLSCLKTLPSFAVCKKVGYRIAELKNLKNLCGTICLSNLENVKDGAEARDAMICDKPYIKRLELEWSRFSRDGSIEMDVLAGLKPDKNLKELQVINYGGSSFPAWLTSPSCMLVSIYMQNCRQDDFLPSLGQLPFLKTLHVEGMHSVKYVDYHFCGESTTGAFPSLESLKIQDMMCLMSWYPLSDNSLLQLRDLTIEDCPSLFSMQSLKHMSSLQELVINCCPGLETLPQLPGSVQSLIIFGSDMVKQRCQIEEGPEWNMIKTIPYVEIDYESMFPGDSS

SEQ ID NO: 5 - DNA, 141 bp, Artificial Sequence
  Marker s3e4516s05
  misc_feature (71)..(71): single nucleotide polymorphism: resistant: c (cytosine); sensitive: t (thymine)
agcacccaaacctccgagarmycacccgatcactccaacyccccatykccctcttcgccrccgccaacganacaaccaccgcaagccccacaagaaagaaagcctcacaaggcaatggacgcggtrgaaytaagrcgggtg

SEQ ID NO: 6 - DNA, 141 bp, Artificial Sequence
  Marker s3e5918s01
  misc_feature (71)..(71): single nucleotide polymorphism: resistant: a (adenine); sensitive: g (guanine)
taagagattawgtgtattaraatctccgacctcatagtatcttaaagagccaaatctccataacggagtcnatagcaacaaacctasatattgtaggtaatatctctctaagccagaaggaacacttatagagtgtagagg